European Patent Specification EP 3 902 837 B1, published March 5, 2025. Title: Monoclonal Antibody Against Human Interleukin-4 Receptor Alpha and Use Thereof. Applicant: Qyuns Therapeutics Co., Ltd. The sequence listing filed with the application follows.

SEQUENCE LISTING (21 sequences)

SEQ ID NO: 1 - protein, 5 aa, Artificial Sequence
TNSMS

SEQ ID NO: 2 - protein, 16 aa, Artificial Sequence
IIGSSGYMDYASWAKG

SEQ ID NO: 3 - protein, 9 aa, Artificial Sequence
HGDSSSFAL

SEQ ID NO: 4 - protein, 13 aa, Artificial Sequence
RASESVYKNNRLS

SEQ ID NO: 5 - protein, 7 aa, Artificial Sequence
EASKVAS

SEQ ID NO: 6 - protein, 10 aa, Artificial Sequence
AGAYRGNIYP

SEQ ID NO: 7 - protein, 117 aa, Artificial Sequence
EVQLVESGGGLVQPGGSLRLSCAASGIDLRTNSMSWVRQAPGKGLEWVGIIGSSGYMDYASWAKGRFTISRDNSKNTLYLQMNSLRAEDTAVYYCARHGDSSSFALWGQGTLVTVSS

SEQ ID NO: 8 - protein, 110 aa, Artificial Sequence
DIQMTQSPSSLSASVGDRVTITCRASESVYKNNRLSWYQQKPGKAPKLLIYEASKVASGVPSRFSGSGSGTDFTLTISSLQPEDFATYYCAGAYRGNIYPFGQGTKVEIK

SEQ ID NO: 9 - protein, 232 aa, Artificial Sequence
MGWLCSGLLFPVSCLVLLQVASSGNMKVLQEPTCVSDYMSISTCEWKMNGPTNCSTELRLLYQLVFLLSEAHTCIPENNGGAGCVCHLLMDDVVSADNYTLDLWAGQQLLWKGSFKPSEHVKPRAPGNLTVHTNVSDTLLLTWSNPYPPDNYLYNHLTYAVNIWSENDPADFRIYNVTYLEPSLRIAASTLKSGISYRARVRAWAQCYNTTWSEWSPSTKWHNSYREPFEQH

SEQ ID NO: 10 - protein, 444 aa, Artificial Sequence
EVQLVESGGGLVQPGGSLRLSCAASGIDLRTNSMSWVRQAPGKGLEWVGIIGSSGYMDYASWAKGRFTISRDNSKNTLYLQMNSLRAEDTAVYYCARHGDSSSFALWGQGTLVTVSSASTKGPSVFPLAPCSRSTSESTAALGCLVKDYFPEPVTVSWNSGALTSGVHTFPAVLQSSGLYSLSSVVTVPSSSLGTKTYTCNVDHKPSNTKVDKRVESKYGPPCPPCPAPEFLGGPSVFLFPPKPKDTLMISRTPEVTCVVVDVSQEDPEVQFNWYVDGVEVHNAKTKPREEQFNSTYRVVSVLTVLHQDWLNGKEYKCKVSNKGLPSSIEKTISKAKGQPREPQVYTLPPSQEEMTKNQVSLTCLVKGFYPSDIAVEWESNGQPENNYKTTPPVLDSDGSFFLYSRLTVDKSRWQEGNVFSCSVMHEALHNHYTQKSLSLSLGK

SEQ ID NO: 11 - protein, 217 aa, Artificial Sequence
DIQMTQSPSSLSASVGDRVTITCRASESVYKNNRLSWYQQKPGKAPKLLIYEASKVASGVPSRFSGSGSGTDFTLTISSLQPEDFATYYCAGAYRGNIYPFGQGTKVEIKRTVAAPSVFIFPPSDEQLKSGTASVVCLLNNFYPREAKVQWKVDNALQSGNSQESVTEQDSKDSTYSLSSTLTLSKADYEKHKVYACEVTHQGLSSPVTKSFNRGEC

SEQ ID NO: 12 - protein, 116 aa, Artificial Sequence
EVQLVESGGGLVQPGGSLRLSCAASGFSLNSNAVGWVRQAPGKGLEYIGFINFSGITYYANWAKGRFTISRDNSKNTLYLQMNSLRAEDTAVYYCARGSAGSFDLWGQGTLVTVSS

SEQ ID NO: 13 - protein, 110 aa, Artificial Sequence
DIQMTQSPSSLSASVGDRVTITCQASESVYKNNYLAWYQQKPGKAPKLLIYRASNLASGVPSRFSGSGSGTDFTLTISSLQPEDFATYYCQGGYSSGMYPFGQGTKVEIK

SEQ ID NO: 14 - protein, 5 aa, Artificial Sequence
SNAVG

SEQ ID NO: 15 - protein, 16 aa, Artificial Sequence
FINFSGITYYANWAKG

SEQ ID NO: 16 - protein, 8 aa, Artificial Sequence
GSAGSFDL

SEQ ID NO: 17 - protein, 13 aa, Artificial Sequence
QASESVYKNNYLA

SEQ ID NO: 18 - protein, 7 aa, Artificial Sequence
RASNLAS

SEQ ID NO: 19 - protein, 10 aa, Artificial Sequence
QGGYSSGMYP

SEQ ID NO: 20 - protein, 443 aa, Artificial Sequence
EVQLVESGGGLVQPGGSLRLSCAASGFSLNSNAVGWVRQAPGKGLEYIGFINFSGITYYANWAKGRFTISRDNSKNTLYLQMNSLRAEDTAVYYCARGSAGSFDLWGQGTLVTVSSASTKGPSVFPLAPCSRSTSESTAALGCLVKDYFPEPVTVSWNSGALTSGVHTFPAVLQSSGLYSLSSVVTVPSSSLGTKTYTCNVDHKPSNTKVDKRVESKYGPPCPPCPAPEFLGGPSVFLFPPKPKDTLMISRTPEVTCVVVDVSQEDPEVQFNWYVDGVEVHNAKTKPREEQFNSTYRVVSVLTVLHQDWLNGKEYKCKVSNKGLPSSIEKTISKAKGQPREPQVYTLPPSQEEMTKNQVSLTCLVKGFYPSDIAVEWESNGQPENNYKTTPPVLDSDGSFFLYSRLTVDKSRWQEGNVFSCSVMHEALHNHYTQKSLSLSLGK

SEQ ID NO: 21 - protein, 217 aa, Artificial Sequence
DIQMTQSPSSLSASVGDRVTITCQASESVYKNNYLAWYQQKPGKAPKLLIYRASNLASGVPSRFSGSGSGTDFTLTISSLQPEDFATYYCQGGYSSGMYPFGQGTKVEIKRTVAAPSVFIFPPSDEQLKSGTASVVCLLNNFYPREAKVQWKVDNALQSGNSQESVTEQDSKDSTYSLSSTLTLSKADYEKHKVYACEVTHQGLSSPVTKSFNRGEC